European Patent Application EP 4 219 552 A2, published August 2, 2023. Title: IL-11R BINDING PROTEINS AND USES THEREOF. Applicant: CSL Limited. Application EP. The sequence listing filed with the application follows.

SEQUENCE LISTING (110 sequences)

SEQ ID NO: 1 - protein, 422 aa, Homo sapiens
MSSSCSGLSRVLVAVATALVSASSPCPQAWGPPGVQYGQPGRSVKLCCPGVTAGDPVSWFRDGEPKLLQGPDSGLGHELVLAQADSTDEGTYICQTLDGALGGTVTLQLGYPPARPVVSCQAADYENFSCTWSPSQISGLPTRYLTSYRKKTVLGADSQRRSPSTGPWPCPQDPLGAARCVVHGAEFWSQYRINVTEVNPLGASTRLLDVSLQSILRPDPPQGLRVESVPGYPRRLRASWTYPASWPCQPHFLLKFRLQYRPAQHPAWSTVEPAGLEEVITDAVAGLPHAVRVSARDFLDAGTWSTWSPEAWGTPSTGTIPKEIPAWGQLHTQPEVEPQVDSPAPPRPSLQPHPRLLDHRDSVEQVAVLASLGILSFLGLVAGALALGLWLRLRRGGKDGSPKPGFLASVIPVDRRPGAPNL

SEQ ID NO: 2 - protein, 432 aa, Macaca fascicularis
MSSSCSGLTRVLVAVATALVSSSSPCPQAWGPPGVQYGQPGRPVMLCCPGVSAGTPVSWFRDGDSRLLQGPDSGLGHRLVLAQVDSPDEGTYVCQTLDGVSGGMVTLKLGFPPARPEVSCQAVDYENFSCTWSPGQVSGLPTRYLTSYRKKTLPGAESQRESPSTGPWPCPQDPLEASRCVVHGAEFWSEYRINVTEVNPLGASTCLLDVRLQSILRPDPPQGLRVESVPGYPRRLHASWTYPASWRRQPHFLLKFRLQYRPAQHPAWSTVEPIGLEEVITDTVAGLPHAVRVSARDFLDAGTWSAWSPEAWGTPSTGLLQDEIPDWSQGHGQQLEAVVAQEDSLAPARPSLQPDPRPLDHRDPLEQVAVLASLGIFSCLGLAVGALALGLWLRLRRSGKEGPQKPGLLAPMIPVEKLPGIPNLQRTPENFS

SEQ ID NO: 3 - protein, 349 aa, synthetic construct
  REGION 1..349: note = polypeptide comprising amino acids 23 to 363 of SEQ ID NO: 1 comprising a 8xHIS tag and a serine at a position corresponding to position 248 of SEQ ID NO: 1 (also referred to as "WT F/L")
SSPCPQAWGPPGVQYGQPGRSVKLCCPGVTAGDPVSWFRDGEPKLLQGPDSGLGHELVLAQADSTDEGTYICQTLDGALGGTVTLQLGYPPARPVVSCQAADYENFSCTWSPSQISGLPTRYLTSYRKKTVLGADSQRRSPSTGPWPCPQDPLGAARCVVHGAEFWSQYRINVTEVNPLGASTRLLDVSLQSILRPDPPQGLRVESVPGYPRRLRASWTYPASWPSQPHFLLKFRLQYRPAQHPAWSTVEPAGLEEVITDAVAGLPHAVRVSARDFLDAGTWSTWSPEAWGTPSTGTIPKEIPAWGQLHTQPEVEPQVDSPAPPRPSLQPHPRLLDHRDSVHHHHHHHH

SEQ ID NO: 4 - protein, 422 aa, Homo sapiens; identical to SEQ ID NO: 1

SEQ ID NO: 5 - protein, 107 aa, synthetic construct
  REGION 1..107: note = amino acid sequence of VL chain of antibody 8E2
DIQMTQSPSSLSASVGDRVTITCQASQDINNYLNWYQQKPGKAPKLLIYDASNLQTGVPSRFSGSGSGTDFTFTISSLQPEDIATYYCQQYDNLSPTFGPGTKVDIK

SEQ ID NO: 6 - protein, 107 aa, synthetic construct
  REGION 1..107: note = amino acid sequence of VL chain of antibody TS-303
DIQMTQSPSSLSASVGDRVTITCQASQDVDYWVEWYQQKPGKAPKLLIYDASNLQTGVPSRFSGSGSGTDFTFTISSLQPEDIATYYCQQYDNLSPTFGPGTKVDIK

SEQ ID NO: 7 - protein, 107 aa, synthetic construct
  REGION 1..107: note = amino acid sequence of VL chain of antibody TS-305
DIQMTQSPSSLSASVGDRVTITCQASQDVGIYVEWYQQKPGKAPKLLIYDASNLQTGVPSRFSGSGSGTDFTFTISSLQPEDIATYYCQQYDNLSPTFGPGTKVDIK

SEQ ID NO: 8 - protein, 107 aa, synthetic construct
  REGION 1..107: note = mino acid sequence of VL chain of antibody TS-306
DIQMTQSPSSLSASVGDRVTITCQASQDVDKYVEWYQQKPGKAPKLLIYDASNLQTGVPSRFSGSGSGTDFTFTISSLQPEDIATYYCQQYDNLSPTFGPGTKVDIK

SEQ ID NO: 9 - protein, 107 aa, synthetic construct
  REGION 1..107: note = amino acid sequence of VL chain of antibody TS-307
DIQMTQSPSSLSASVGDRVTITCQASQDVSMYVEWYQQKPGKAPKLLIYDASNLQTGVPSRFSGSGSGTDFTFTISSLQPEDIATYYCQQYDNLSPTFGPGTKVDIK

SEQ ID NO: 10 - protein, 107 aa, synthetic construct
  REGION 1..107: note = amino acid sequence of VL chain of antibody TS-310
DIQMTQSPSSLSASVGDRVTITCQASQDVAMYIEWYQQKPGKAPKLLIYDASNLQTGVPSRFSGSGSGTDFTFTISSLQPEDIATYYCQQYDNLSPTFGPGTKVDIK

SEQ ID NO: 11 - protein, 107 aa, synthetic construct
  REGION 1..107: note = amino acid sequence of VL chain of antibody TS-311
DIQMTQSPSSLSASVGDRVTITCQASQDVSQYIEWYQQKPGKAPKLLIYDASNLQTGVPSRFSGSGSGTDFTFTISSLQPEDIATYYCQQYDNLSPTFGPGTKVDIK

SEQ ID NO: 12 - protein, 107 aa, synthetic construct
  REGION 1..107: note = amino acid sequence of VL chain of antibody TS-312
DIQMTQSPSSLSASVGDRVTITCQASQDIGQYVEWYQQKPGKAPKLLIYDASNLQTGVPSRFSGSGSGTDFTFTISSLQPEDIATYYCQQYDNLSPTFGPGTKVDIK

SEQ ID NO: 13 - protein, 107 aa, synthetic construct
  REGION 1..107: note = amino acid sequence of VL chain of antibody TS-313
DIQMTQSPSSLSASVGDRVTITCQASQDVSGYVEWYQQKPGKAPKLLIYDASNLQTGVPSRFSGSGSGTDFTFTISSLQPEDIATYYCQQYDNLSPTFGPGTKVDIK

SEQ ID NO: 14 - protein, 107 aa, synthetic construct
  REGION 1..107: note = amino acid sequence of VL chain of antibody TS-322
DIQMTQSPSSLSASVGDRVTITCQASQDVHHYMEWYQQKPGKAPKLLIYDASNLQTGVPSRFSGSGSGTDFTFTISSLQPEDIATYYCQQYDNLSPTFGPGTKVDIK

SEQ ID NO: 15 - protein, 107 aa, synthetic construct
  REGION 1..107: note = amino acid sequence of VL chain of antibody TS-2
DIQMTQSPSSLSASVGDRVTITCQASQDINNYLNWYQQKPGKAPKLLIYDASNLQTGVPSRFSGSGSGTDFTFTISSLQPEDIATYYCQQAEDQSPTFGPGTKVDIK

SEQ ID NO: 16 - protein, 107 aa, synthetic construct
  REGION 1..107: note = amino acid sequence of VL chain of antibody TS-4
DIQMTQSPSSLSASVGDRVTITCQASQDINNYLNWYQQKPGKAPKLLIYDASNLQTGVPSRFSGSGSGTDFTFTISSLQPEDIATYYCQQHEFQSPTFGPGTKVDIK

SEQ ID NO: 17 - protein, 107 aa, synthetic construct
  REGION 1..107: note = amino acid sequence of VL chain of antibody TS-6
DIQMTQSPSSLSASVGDRVTITCQASQDINNYLNWYQQKPGKAPKLLIYDASNLQTGVPSRFSGSGSGTDFTFTISSLQPEDIATYYCEQFESQSPTFGPGTKVDIK

SEQ ID NO: 18 - protein, 107 aa, synthetic construct
  REGION 1..107: note = amino acid sequence of VL chain of antibody TS-7
DIQMTQSPSSLSASVGDRVTITCQASQDINNYLNWYQQKPGKAPKLLIYDASNLQTGVPSRFSGSGSGTDFTFTISSLQPEDIATYYCQQHENQSPTFGPGTKVDIK

SEQ ID NO: 19 - protein, 107 aa, synthetic construct
  REGION 1..107: note = amino acid sequence of VL chain of antibody TS-9
DIQMTQSPSSLSASVGDRVTITCQASQDINNYLNWYQQKPGKAPKLLIYDASNLQTGVPSRFSGSGSGTDFTFTISSLQPEDIATYYCQQAEEQSPTFGPGTKVDIK

SEQ ID NO: 20 - protein, 107 aa, synthetic construct
  REGION 1..107: note = amino acid sequence of VL chain of antibody TS-13
DIQMTQSPSSLSASVGDRVTITCQASQDINNYLNWYQQKPGKAPKLLIYDASNLQTGVPSRFSGSGSGTDFTFTISSLQPEDIATYYCQQNETQSPTFGPGTKVDIK

SEQ ID NO: 21 - protein, 107 aa, synthetic construct
  REGION 1..107: note = amino acid sequence of VL chain of antibody TS-14
DIQMTQSPSSLSASVGDRVTITCQASQDINNYLNWYQQKPGKAPKLLIYDASNLQTGVPSRFSGSGSGTDFTFTISSLQPEDIATYYCQQHDNQSPTFGPGTKVDIK

SEQ ID NO: 22 - protein, 107 aa, synthetic construct
  REGION 1..107: note = amino acid sequence of VL chain of antibody TS-17
DIQMTQSPSSLSASVGDRVTITCQASQDINNYLNWYQQKPGKAPKLLIYDASNLQTGVPSRFSGSGSGTDFTFTISSLQPEDIATYYCSQFESQSPTFGPGTKVDIK

SEQ ID NO: 23 - protein, 107 aa, synthetic construct
  REGION 1..107: note = amino acid sequence of VL chain of antibody TS-20
DIQMTQSPSSLSASVGDRVTITCQASQDINNYLNWYQQKPGKAPKLLIYDASNLQTGVPSRFSGSGSGTDFTFTISSLQPEDIATYYCQQNESQSPTFGPGTKVDIK

SEQ ID NO: 24 - protein, 107 aa, synthetic construct
  REGION 1..107: note = amino acid sequence of VL chain of antibody TS-21
DIQMTQSPSSLSASVGDRVTITCQASQDINNYLNWYQQKPGKAPKLLIYDASNLQTGVPSRFSGSGSGTDFTFTISSLQPEDIATYYCQQSESQSPTFGPGTKVDIK

SEQ ID NO: 25 - protein, 107 aa, synthetic construct
  REGION 1..107: note = amino acid sequence of VL chain of antibody TS-22
DIQMTQSPSSLSASVGDRVTITCQASQDINNYLNWYQQKPGKAPKLLIYDASNLQTGVPSRFSGSGSGTDFTFTISSLQPEDIATYYCQQFETQSPTFGPGTKVDIK

SEQ ID NO: 26 - protein, 107 aa, synthetic construct
  REGION 1..107: note = amino acid sequence of VL chain of antibody TS-29
DIQMTQSPSSLSASVGDRVTITCQASQDINNYLNWYQQKPGKAPKLLIYDASNLQTGVPSRFSGSGSGTDFTFTISSLQPEDIATYYCQQSEEQSPTFGPGTKVDIK

SEQ ID NO: 27 - protein, 107 aa, synthetic construct
  REGION 1..107: note = amino acid sequence of VL chain of antibody TS-32
DIQMTQSPSSLSASVGDRVTITCQASQDINNYLNWYQQKPGKAPKLLIYDASNLQTGVPSRFSGSGSGTDFTFTISSLQPEDIATYYCTQWETQSPTFGPGTKVDIK

SEQ ID NO: 28 - protein, 107 aa, synthetic construct
  REGION 1..107: note = amino acid sequence of VL chain of antibody TS-49
DIQMTQSPSSLSASVGDRVTITCQASQDINNYLNWYQQKPGKAPKLLIYDASNLQTGVPSRFSGSGSGTDFTFTISSLQPEDIATYYCQQYESQAPEFGPGTKVDIK

SEQ ID NO: 29 - protein, 107 aa, synthetic construct
  REGION 1..107: note = amino acid sequence of VL chain of antibody TS-51
DIQMTQSPSSLSASVGDRVTITCQASQDINNYLNWYQQKPGKAPKLLIYDASNLQTGVPSRFSGSGSGTDFTFTISSLQPEDIATYYCQQYESQWPFFGPGTKVDIK

SEQ ID NO: 30 - protein, 107 aa, synthetic construct
  REGION 1..107: note = amino acid sequence of VL chain of antibody TS-55
DIQMTQSPSSLSASVGDRVTITCQASQDINNYLNWYQQKPGKAPKLLIYDASNLQTGVPSRFSGSGSGTDFTFTISSLQPEDIATYYCQQYETQTPAFGPGTKVDIK

SEQ ID NO: 31 - protein, 107 aa, synthetic construct
  REGION 1..107: note = amino acid sequence of VL chain of antibody TS-57
DIQMTQSPSSLSASVGDRVTITCQASQDINNYLNWYQQKPGKAPKLLIYDASNLQTGVPSRFSGSGSGTDFTFTISSLQPEDIATYYCQQYETQMPLFGPGTKVDIK

SEQ ID NO: 32 - protein, 107 aa, synthetic construct
  REGION 1..107: note = amino acid sequence of VL chain of antibody TS-58
DIQMTQSPSSLSASVGDRVTITCQASQDINNYLNWYQQKPGKAPKLLIYDASNLQTGVPSRFSGSGSGTDFTFTISSLQPEDIATYYCQQYETQQPFFGPGTKVDIK

SEQ ID NO: 33 - protein, 107 aa, synthetic construct
  REGION 1..107: note = amino acid sequence of VL chain of antibody TS-63
DIQMTQSPSSLSASVGDRVTITCQASQDINNYLNWYQQKPGKAPKLLIYDASNLQTGVPSRFSGSGSGTDFTFTISSLQPEDIATYYCQQYDTQQPNFGPGTKVDIK

SEQ ID NO: 34 - protein, 107 aa, synthetic construct
  REGION 1..107: note = amino acid sequence of VL chain of antibody TS-64
DIQMTQSPSSLSASVGDRVTITCQASQDINNYLNWYQQKPGKAPKLLIYDASNLQTGVPSRFSGSGSGTDFTFTISSLQPEDIATYYCQQYESQWPQFGPGTKVDIK

SEQ ID NO: 35 - protein, 107 aa, synthetic construct
  REGION 1..107: note = amino acid sequence of consensus of VL chain of 8E2 antibody and derivatives
  VARIANT 29: note = X=I or V
  VARIANT 30: note = X=N or D or G or S or A or H
  VARIANT 31: note = X=N or Y or I or K or M or Q or G or H
  VARIANT 32: note = X=Y or W
  VARIANT 33: note = X=L or V or I or M
  VARIANT 34: note = X=N or E
  VARIANT 89: note = X=Q or E or S or T
  VARIANT 91: note = X=Y or A or H or F or N or S or W
  VARIANT 92: note = X=D or E
  VARIANT 93: note = X=N or D or F or S or E or T
  VARIANT 94: note = X=L or Q
  VARIANT 95: note = X=S or A or W or T or M or Q
  VARIANT 97: note = X=T or E or F or A or L or N or Q
DIQMTQSPSSLSASVGDRVTITCQASQDXXXXXXWYQQKPGKAPKLLIYDASNLQTGVPSRFSGSGSGTDFTFTISSLQPEDIATYYCXQXXXXXPXFGPGTKVDIK

SEQ ID NO: 36 - protein, 107 aa, synthetic construct
  REGION 1..107: note = amino acid sequence of consensus of VL chain of 8E2 antibody and select derivatives
  VARIANT 29: note = X=I or V
  VARIANT 30: note = X=D or N
  VARIANT 31: note = X=K or N
  VARIANT 33: note = X=L or V
  VARIANT 34: note = X=N or E
  VARIANT 91: note = X=Y or A or H
  VARIANT 92: note = X=D or E
  VARIANT 93: note = X=N or D or F or N or S
  VARIANT 94: note = X=L or Q
  VARIANT 95: note = X=S or W
  VARIANT 97: note = X=T or F
DIQMTQSPSSLSASVGDRVTITCQASQDXXXYXXWYQQKPGKAPKLLIYDASNLQTGVPSRFSGSGSGTDFTFTISSLQPEDIATYYCQQXXXXXPXFGPGTKVDIK

SEQ ID NO: 37 - protein, 118 aa, synthetic construct
  REGION 1..118: note = amino acid sequence of VH chain of antibody 8E2
EVQLLESGGGLVQPGGSLRLSCAASGFTFSWYSMTWVRQAPGKGLEWVSSIVPSGGHTQYADSVKGRFTISRDNSKNTLYLQMNSLRAEDTAVYYCAKGPGWGSFDLWGRGTLVTVSS

SEQ ID NO: 38 - protein, 118 aa, synthetic construct
  REGION 1..118: note = amino acid sequence of VH chain of antibody TS-66
EVQLLESGGGLVQPGGSLRLSCAASGFTFAWWSIAWVRQAPGKGLEWVSSIVPSGGHTQYADSVKGRFTISRDNSKNTLYLQMNSLRAEDTAVYYCAKGPGWGSFDLWGRGTLVTVSS

SEQ ID NO: 39 - protein, 118 aa, synthetic construct
  REGION 1..118: note = amino acid sequence of VH chain of antibody TS-69
EVQLLESGGGLVQPGGSLRLSCAASGFTFGWWSVTWVRQAPGKGLEWVSSIVPSGGHTQYADSVKGRFTISRDNSKNTLYLQMNSLRAEDTAVYYCAKGPGWGSFDLWGRGTLVTVSS

SEQ ID NO: 40 - protein, 118 aa, synthetic construct
  REGION 1..118: note = amino acid sequence of VH chain of antibody TS-71
EVQLLESGGGLVQPGGSLRLSCAASGFTFWRWSTTWVRQAPGKGLEWVSSIVPSGGHTQYADSVKGRFTISRDNSKNTLYLQMNSLRAEDTAVYYCAKGPGWGSFDLWGRGTLVTVSS

SEQ ID NO: 41 - protein, 118 aa, synthetic construct
  REGION 1..118: note = amino acid sequence of VH chain of antibody TS-76
EVQLLESGGGLVQPGGSLRLSCAASGFTFWRWSITWVRQAPGKGLEWVSSIVPSGGHTQYADSVKGRFTISRDNSKNTLYLQMNSLRAEDTAVYYCAKGPGWGSFDLWGRGTLVTVSS

SEQ ID NO: 42 - protein, 118 aa, synthetic construct
  REGION 1..118: note = amino acid sequence of VH chain of antibody TS-79
EVQLLESGGGLVQPGGSLRLSCAASGFTFAWFSVTWVRQAPGKGLEWVSSIVPSGGHTQYADSVKGRFTISRDNSKNTLYLQMNSLRAEDTAVYYCAKGPGWGSFDLWGRGTLVTVSS

SEQ ID NO: 43 - protein, 118 aa, synthetic construct
  REGION 1..118: note = amino acid sequence of VH chain of antibody TS-82
EVQLLESGGGLVQPGGSLRLSCAASGFTFWRWSVTWVRQAPGKGLEWVSSIVPSGGHTQYADSVKGRFTISRDNSKNTLYLQMNSLRAEDTAVYYCAKGPGWGSFDLWGRGTLVTVSS

SEQ ID NO: 44 - protein, 118 aa, synthetic construct; identical to SEQ ID NO: 40
  REGION 1..118: note = amino acid sequence of VH chain of antibody TS-88

SEQ ID NO: 45 - protein, 118 aa, synthetic construct; identical to SEQ ID NO: 41
  REGION 1..118: note = amino acid sequence of VH chain of antibody TS-89

SEQ ID NO: 46 - protein, 118 aa, synthetic construct
  REGION 1..118: note = amino acid sequence of VH chain of antibody TS-91
EVQLLESGGGLVQPGGSLRLSCAASGFTFGWWSLTWVRQAPGKGLEWVSSIVPSGGHTQYADSVKGRFTISRDNSKNTLYLQMNSLRAEDTAVYYCAKGPGWGSFDLWGRGTLVTVSS

SEQ ID NO: 47 - protein, 118 aa, synthetic construct
  REGION 1..118: note = amino acid sequence of VH chain of antibody TS-92
EVQLLESGGGLVQPGGSLRLSCAASGFTFSWWSITWVRQAPGKGLEWVSSIVPSGGHTQYADSVKGRFTISRDNSKNTLYLQMNSLRAEDTAVYYCAKGPGWGSFDLWGRGTLVTVSS

SEQ ID NO: 48 - protein, 118 aa, synthetic construct
  REGION 1..118: note = amino acid sequence of VH chain of antibody TS-97
EVQLLESGGGLVQPGGSLRLSCAASGFTFSWYSMTWVRQAPGKGLEWVSSIVPWADYTQYADSVKGRFTISRDNSKNTLYLQMNSLRAEDTAVYYCAKGPGWGSFDLWGRGTLVTVSS

SEQ ID NO: 49 - protein, 118 aa, synthetic construct
  REGION 1..118: note = amino acid sequence of VH chain of antibody TS-101
EVQLLESGGGLVQPGGSLRLSCAASGFTFSWYSMTWVRQAPGKGLEWVSSIVPWGDLTQYADSVKGRFTISRDNSKNTLYLQMNSLRAEDTAVYYCAKGPGWGSFDLWGRGTLVTVSS

SEQ ID NO: 50 - protein, 118 aa, synthetic construct
  REGION 1..118: note = amino acid sequence of VH chain of antibody TS-103
EVQLLESGGGLVQPGGSLRLSCAASGFTFSWYSMTWVRQAPGKGLEWVSSIVPYGDLTQYADSVKGRFTISRDNSKNTLYLQMNSLRAEDTAVYYCAKGPGWGSFDLWGRGTLVTVSS

SEQ ID NO: 51 - protein, 118 aa, synthetic construct
  REGION 1..118: note = amino acid sequence of VH chain of antibody TS-104
EVQLLESGGGLVQPGGSLRLSCAASGFTFSWYSMTWVRQAPGKGLEWVSSIVPWGTITQYADSVKGRFTISRDNSKNTLYLQMNSLRAEDTAVYYCAKGPGWGSFDLWGRGTLVTVSS

SEQ ID NO: 52 - protein, 118 aa, synthetic construct
  REGION 1..118: note = amino acid sequence of VH chain of antibody TS-107
EVQLLESGGGLVQPGGSLRLSCAASGFTFSWYSMTWVRQAPGKGLEWVSSIVPWGDFTQYADSVKGRFTISRDNSKNTLYLQMNSLRAEDTAVYYCAKGPGWGSFDLWGRGTLVTVSS

SEQ ID NO: 53 - protein, 118 aa, synthetic construct
  REGION 1..118: note = amino acid sequence of VH chain of antibody TS-108
EVQLLESGGGLVQPGGSLRLSCAASGFTFSWYSMTWVRQAPGKGLEWVSSIVPWGTLTQYADSVKGRFTISRDNSKNTLYLQMNSLRAEDTAVYYCAKGPGWGSFDLWGRGTLVTVSS

SEQ ID NO: 54 - protein, 118 aa, synthetic construct
  REGION 1..118: note = amino acid sequence of VH chain of antibody TS-115
EVQLLESGGGLVQPGGSLRLSCAASGFTFSWYSMTWVRQAPGKGLEWVSSIVPHGDLTQYADSVKGRFTISRDNSKNTLYLQMNSLRAEDTAVYYCAKGPGWGSFDLWGRGTLVTVSS

SEQ ID NO: 55 - protein, 118 aa, synthetic construct
  REGION 1..118: note = amino acid sequence of VH chain of antibody TS-129
EVQLLESGGGLVQPGGSLRLSCAASGFTFSWYSMTWVRQAPGKGLEWVSSIVPSGGHTQYADSVKGRFTISRDNSKNTLYLQMNSLRAEDTAVYYCAKPEDWGMFDLWGRGTLVTVSS

SEQ ID NO: 56 - protein, 118 aa, synthetic construct
  REGION 1..118: note = amino acid sequence of VH chain of antibody TS-133
EVQLLESGGGLVQPGGSLRLSCAASGFTFSWYSMTWVRQAPGKGLEWVSSIVPSGGHTQYADSVKGRFTISRDNSKNTLYLQMNSLRAEDTAVYYCAKPVDWGRFDLWGRGTLVTVSS

SEQ ID NO: 57 - protein, 118 aa, synthetic construct
  REGION 1..118: note = amino acid sequence of VH chain of antibody TS-134
EVQLLESGGGLVQPGGSLRLSCAASGFTFSWYSMTWVRQAPGKGLEWVSSIVPSGGHTQYADSVKGRFTISRDNSKNTLYLQMNSLRAEDTAVYYCAKPEDWGLFDLWGRGTLVTVSS

SEQ ID NO: 58 - protein, 118 aa, synthetic construct
  REGION 1..118: note = amino acid sequence of VH chain of antibody TS-135
EVQLLESGGGLVQPGGSLRLSCAASGFTFSWYSMTWVRQAPGKGLEWVSSIVPSGGHTQYADSVKGRFTISRDNSKNTLYLQMNSLRAEDTAVYYCAKPLDWGLFDLWGRGTLVTVSS

SEQ ID NO: 59 - protein, 118 aa, synthetic construct
  REGION 1..118: note = amino acid sequence of VH chain of antibody TS-136
EVQLLESGGGLVQPGGSLRLSCAASGFTFSWYSMTWVRQAPGKGLEWVSSIVPSGGHTQYADSVKGRFTISRDNSKNTLYLQMNSLRAEDTAVYYCAKPLDWGRFDLWGRGTLVTVSS

SEQ ID NO: 60 - protein, 118 aa, synthetic construct
  REGION 1..118: note = amino acid sequence of VH chain of antibody TS-140
EVQLLESGGGLVQPGGSLRLSCAASGFTFSWYSMTWVRQAPGKGLEWVSSIVPSGGHTQYADSVKGRFTISRDNSKNTLYLQMNSLRAEDTAVYYCAKPNDWGLFDLWGRGTLVTVSS

SEQ ID NO: 61 - protein, 118 aa, synthetic construct
  REGION 1..118: note = amino acid sequence of VH chain of antibody TS-143
EVQLLESGGGLVQPGGSLRLSCAASGFTFSWYSMTWVRQAPGKGLEWVSSIVPSGGHTQYADSVKGRFTISRDNSKNTLYLQMNSLRAEDTAVYYCAKPHDWGLFDLWGRGTLVTVSS

SEQ ID NO: 62 - protein, 118 aa, synthetic construct
  REGION 1..118: note = amino acid sequence of VH chain of antibody TS-151
EVQLLESGGGLVQPGGSLRLSCAASGFTFSWYSMTWVRQAPGKGLEWVSSIVPSGGHTQYADSVKGRFTISRDNSKNTLYLQMNSLRAEDTAVYYCAKPHDWGRFDLWGRGTLVTVSS

SEQ ID NO: 63 - protein, 118 aa, synthetic construct
  REGION 1..118: note = amino acid sequence of VH chain of antibody TS-156
EVQLLESGGGLVQPGGSLRLSCAASGFTFSWYSMTWVRQAPGKGLEWVSSIVPSGGHTQYADSVKGRFTISRDNSKNTLYLQMNSLRAEDTAVYYCAKPEDWGRFDLWGRGTLVTVSS

SEQ ID NO: 64 - protein, 118 aa, synthetic construct
  REGION 1..118: note = amino acid sequence of VH chain of antibody TS-213
EVQLLESGGGLVQPGGSLRLSCAASGFTFSWYSMTWVRQAPGKGLEWVSSIVPSGGHTQYADSVKGRFTISRDNSKNTLYLQMNSLRAEDTAVYYCAKGPGWGQFAVWGRGTLVTVSS

SEQ ID NO: 65 - protein, 118 aa, synthetic construct
  REGION 1..118: note = amino acid sequence of VH chain of antibody TS-214
EVQLLESGGGLVQPGGSLRLSCAASGFTFSWYSMTWVRQAPGKGLEWVSSIVPSGGHTQYADSVKGRFTISRDNSKNTLYLQMNSLRAEDTAVYYCAKGPGWGSFWFWGRGTLVTVSS

SEQ ID NO: 66 - protein, 118 aa, synthetic construct
  REGION 1..118: note = amino acid sequence of VH chain of antibody TS-215
EVQLLESGGGLVQPGGSLRLSCAASGFTFSWYSMTWVRQAPGKGLEWVSSIVPSGGHTQYADSVKGRFTISRDNSKNTLYLQMNSLRAEDTAVYYCAKGPGWGSFWQWGRGTLVTVSS

SEQ ID NO: 67 - protein, 118 aa, synthetic construct
  REGION 1..118: note = amino acid sequence of VH chain of antibody TS-218
EVQLLESGGGLVQPGGSLRLSCAASGFTFSWYSMTWVRQAPGKGLEWVSSIVPSGGHTQYADSVKGRFTISRDNSKNTLYLQMNSLRAEDTAVYYCAKGPGWGSFWEWGRGTLVTVSS

SEQ ID NO: 68 - protein, 118 aa, synthetic construct
  REGION 1..118: note = amino acid sequence of VH chain of antibody TS-221
EVQLLESGGGLVQPGGSLRLSCAASGFTFSWYSMTWVRQAPGKGLEWVSSIVPSGGHTQYADSVKGRFTISRDNSKNTLYLQMNSLRAEDTAVYYCAKGPGWGSFWYWGRGTLVTVSS

SEQ ID NO: 69 - protein, 118 aa, synthetic construct
  REGION 1..118: note = amino acid sequence of VH chain of antibody TS-222
EVQLLESGGGLVQPGGSLRLSCAASGFTFSWYSMTWVRQAPGKGLEWVSSIVPSGGHTQYADSVKGRFTISRDNSKNTLYLQMNSLRAEDTAVYYCAKGPGWGTFAYWGRGTLVTVSS

SEQ ID NO: 70 - protein, 118 aa, synthetic construct
  REGION 1..118: note = amino acid sequence of VH chain of antibody TS-224
EVQLLESGGGLVQPGGSLRLSCAASGFTFSWYSMTWVRQAPGKGLEWVSSIVPSGGHTQYADSVKGRFTISRDNSKNTLYLQMNSLRAEDTAVYYCAKGPGWGSFWTWGRGTLVTVSS

SEQ ID NO: 71 - protein, 118 aa, synthetic construct
  REGION 1..118: note = amino acid sequence of consensus of VH chain of 8E2 antibody and derivatives
  VARIANT 30: note = X= any naturally occurring amino acid
  VARIANT 31: note = X=W or R
  VARIANT 32: note = X=Y or W or F
  VARIANT 34: note = X=M or I or V or T or L
  VARIANT 35: note = X=T or A
  VARIANT 53: note = X=S or W or Y or H
  VARIANT 54: note = X=G or A
  VARIANT 55: note = X=G or D or T
  VARIANT 56: note = X=H or Y or L or I or F
  VARIANT 99: note = X=G or P
  VARIANT 100: note = X=P or E or V or L or N or H or E
  VARIANT 101: note = X=G or D
  VARIANT 104: note = X=S or M or R or L or Q or T
  VARIANT 106: note = X=D or A or W
  VARIANT 107: note = X=L or V or F or Q or E or Y or T
  VARIANT 57: note = X= any naturally occurring amino acid
EVQLLESGGGLVQPGGSLRLSCAASGFTFXXXSXXWVRQAPGKGLEWVSSIVPXXXXTQYADSVKGRFTISRDNSKNTLYLQMNSLRAEDTAVYYCAKXXXWGXFXXWGRGTLVTVSS

SEQ ID NO: 72 - protein, 118 aa, synthetic construct
  REGION 1..118: note = amino acid sequence of consensus of VH chain of 8E2 antibody and select derivatives
  VARIANT 53: note = X=W or S
  VARIANT 55: note = X=G or D or T
  VARIANT 56: note = X=H or L
  VARIANT 99: note = X=G or P
  VARIANT 100: note = X=P or E or L
  VARIANT 101: note = X=G or D
  VARIANT 104: note = X=S or L or R
  VARIANT 54: note = X= any naturally occurring amino acid
  VARIANT 57: note = X= any naturally occurring amino acid
EVQLLESGGGLVQPGGSLRLSCAASGFTFSWYSMTWVRQAPGKGLEWVSSIVPXGXXTQYADSVKGRFTISRDNSKNTLYLQMNSLRAEDTAVYYCAKXXXWGXFDLWGRGTLVTVSS

SEQ ID NO: 73 - protein, 114 aa, synthetic construct
  REGION 1..114: note = amino acid sequence of VL chain of antibody 8E4
QSALTQPPSASGSPGQSVAISCTGTSSDVGGYNFVSWYQQHPGKAPKLLIYEVTKRPSGVPDRFSGSKAGNTASLTVSGLQAEDEADYYCSSYGGSNNAGVFGTGTKVTVLGQP

SEQ ID NO: 74 - protein, 126 aa, synthetic construct
  REGION 1..126: note = amino acid sequence of VH chain of antibody 8E4
EVQLLESGGGLVQPGGSLRLSCAASGFTFSWYFMGWVRQAPGKGLEWVSYIYPSGGSTGYADSVKGRFTISRDNSKNTLYLQMHSLRAEDTAVYYCARDEGYCSSTSCYFDAFDIWGQGTMVTVSS

SEQ ID NO: 75 - protein, 107 aa, synthetic construct
  REGION 1..107: note = amino acid sequence of VL chain of antibody 8D10
DIQMTQSPSSLSASVGDRVTITCQASQDITNYLNWYLHKPGKAPKLLIYDASNLQTGVPSRFSGSGSGTDFTFTITSLQPEDFGTYYCQQYDTLHPSFGPGTTVDIK

SEQ ID NO: 76 - protein, 118 aa, synthetic construct
  REGION 1..118: note = amino acid sequence of VH chain of antibody 8D10
EVQLLESGGGLVQPGGSLRLSCAASGFTFSRYMMGWVRQAPGKGLEWVSSIVPSGGITIYADSVKGRFTISRDNSKNTLYLQMNSLRAEDTAVYYCARDHMGIVATDWGQGTLVTVSS

SEQ ID NO: 77 - protein, 11 aa, synthetic construct
  REGION 1..11: note = amino acid sequence of consensus of CDR1 of VL chain of 8E2 antibody and derivatives
  VARIANT 6: note = X=I or V
  VARIANT 7: note = X=N or D or G or S or A or H
  VARIANT 8: note = X=N or Y or I or K or M or Q or G or H
  VARIANT 9: note = X=Y or W
  VARIANT 10: note = X=L or V or I or M
  VARIANT 11: note = X=N or E
QASQDXXXXXX

SEQ ID NO: 78-79 - skipped (2 entries)

SEQ ID NO: 80 - protein, 17 aa, synthetic construct
  REGION 1..17: note = amino acid sequence of consensus of CDR2 of VH chain of 8E2 antibody and derivatives
  VARIANT 5: note = X=S or W or Y or H
  VARIANT 6: note = X=G or A
  VARIANT 7: note = X=G or D or T
  VARIANT 8: note = X=H or Y or L or I or F
SIVPXXXXTQYADSVKG

SEQ ID NO: 81 - skipped

SEQ ID NO: 82 - protein, 424 aa, Mus musculus
MSSSCSGLTRVLVAVATALVSSSSPCPQAWGPPGVQYGQPGRPVMLCCPGVSAGTPVSWFRDGDSRLLQGPDSGLGHRLVLAQVDSPDEGTYVCQTLDGVSGGMVTLKLGFPPARPEVSCQAVDYENFSCTWSPGQVSGLPTRYLTSYRKKTLPGAESQRESPSTGPWPCPQDPLEASRCVVHGAEFWSEYRINVTEVNPLGASTCLLDVRLQSILRPDPPQGLRVESVPGYPRRLHASWTYPASWRRQPHFLLKFRLQYRPAQHPAWSTVEPIGLEEVITDTVAGLPHAVRVSARDFLDAGTWSAWSPEAWGTPSTGLLQDEIPDWSQGHGQQLEAVVAQEDSLAPARPSLQPDPRPLDHRDPLEQVAVLASLGIFSCLGLAVGALALGLWLRLRRSGKEGPQKPGLLAPMIPVEKLPGIPNL

SEQ ID NO: 83 - protein, 214 aa, synthetic construct
  REGION 1..214: note = amino acid sequence of light chain of antibody 8E2
DIQMTQSPSSLSASVGDRVTITCQASQDINNYLNWYQQKPGTAPKLLIYDASNLQTGVPSRFSGSGSGTHFTFTINTLQPEDIATYYCQQYDNLSPTFGPGTKVDIKRTVAAPSVFIFPPSDEQLKSGTASVVCLLNNFYPREAKVQWKVDNALQSGNSQESVTEQDSKDSTYSLSSTLTLSKADYEKHKVYACEVTHQGLSSPVTKSFNRGEC

SEQ ID NO: 84 - protein, 302 aa, synthetic construct
  REGION 1..302: note = amino acid sequence of heavy chain of antibody 8E2
EVQLLESGGGLVQPGGSLRLSCAASGFTFSWYSMTWVRQAPGKGLEWVSSIVPSGGHTQYADSVKGRFTISRDNSKNTLYLQMNSLRAEDTAVYYCAKGPGWGSFDLWGRGTLVTVSSASTKGPSVFPLAPCSRSTSESTAALGCLVKDYFPEPVTVSWNSGALTSGVHTFPAVLQSSGLYSLSSVVTVPSSSLGTKTYTCNVDHKPSNTKVDKRVESKYGPPCPPCPAPEFLGGPSVFLFPPKPKDTLMISRTPEVTCVVVDVSQEDPEVQFNWYVDGVEVHNAKTKPREEQFNSTYRVVS

SEQ ID NO: 85 - protein, 304 aa, synthetic construct
  REGION 1..304: note = polypeptide comprising amino acids 23 to 318 of Homo sapiens IL-11R? (SEQ ID NO: 1), a 8xHIS tag and a serine at a position corresponding to position 248 of SEQ ID NO:1 (also referred to as "WT D1/2")
SSPCPQAWGPPGVQYGQPGRSVKLCCPGVTAGDPVSWFRDGEPKLLQGPDSGLGHELVLAQADSTDEGTYICQTLDGALGGTVTLQLGYPPARPVVSCQAADYENFSCTWSPSQISGLPTRYLTSYRKKTVLGADSQRRSPSTGPWPCPQDPLGAARCVVHGAEFWSQYRINVTEVNPLGASTRLLDVSLQSILRPDPPQGLRVESVPGYPRRLRASWTYPASWPSQPHFLLKFRLQYRPAQHPAWSTVEPAGLEEVITDAVAGLPHAVRVSARDFLDAGTWSTWSPEAWGTPSTGHHHHHHHH

SEQ ID NO: 86 - protein, 353 aa, synthetic construct
  REGION 1..353: note = amino acid sequence of a polypeptide comprising amino acids 23-110 of SEQ ID NO: 1 and amino acids 111-367 of SEQ ID NO: 82 in which there is a serine at a position corresponding to position 206 of SEQ ID NO: 82 and a HIS tag
SSPCPQAWGPPGVQYGQPGRSVKLCCPGVTAGDPVSWFRDGEPKLLQGPDSGLGHELVLAQADSTDEGTYICQTLDGALGGTVTLQLGFPPARPEVSCQAVDYENFSCTWSPGQVSGLPTRYLTSYRKKTLPGAESQRESPSTGPWPCPQDPLEASRCVVHGAEFWSEYRINVTEVNPLGASTSLLDVRLQSILRPDPPQGLRVESVPGYPRRLHASWTYPASWRRQPHFLLKFRLQYRPAQHPAWSTVEPIGLEEVITDAVAGLPHAVRVSARDFLDAGTWSAWSPEAWGTPSTGPLQDEIPDWSQGHGQQLEAVVAQEDSPAPARPSLQPDPRPLDHRDPLEQHHHHHHHH

SEQ ID NO: 87 - protein, 353 aa, synthetic construct
  REGION 1..353: note = amino acid sequence of a polypeptide comprising amino acids 23-215 of SEQ ID NO: 1 and amino acids 216-367 of SEQ ID NO: 82 and a HIS tag
SSPCPQAWGPPGVQYGQPGRSVKLCCPGVTAGDPVSWFRDGEPKLLQGPDSGLGHELVLAQADSTDEGTYICQTLDGALGGTVTLQLGYPPARPVVSCQAADYENFSCTWSPSQISGLPTRYLTSYRKKTVLGADSQRRSPSTGPWPCPQDPLGAARCVVHGAEFWSQYRINVTEVNPLGASTRLLDVSLQSILRPDPPQGLRVESVPGYPRRLHASWTYPASWRRQPHFLLKFRLQYRPAQHPAWSTVEPIGLEEVITDAVAGLPHAVRVSARDFLDAGTWSAWSPEAWGTPSTGPLQDEIPDWSQGHGQQLEAVVAQEDSPAPARPSLQPDPRPLDHRDPLEQHHHHHHHH

SEQ ID NO: 88 - protein, 353 aa, synthetic construct
  REGION 1..353: note = amino acid sequence of a polypeptide comprising amino acids 23-318 of SEQ ID NO: 1 in which there is a serine at a position corresponding to position 226 of SEQ ID NO: 1 and amino acids 319-367 of SEQ ID NO: 82 and a HIS tag
SSPCPQAWGPPGVQYGQPGRSVKLCCPGVTAGDPVSWFRDGEPKLLQGPDSGLGHELVLAQADSTDEGTYICQTLDGALGGTVTLQLGYPPARPVVSCQAADYENFSCTWSPSQISGLPTRYLTSYRKKTVLGADSQRRSPSTGPWPCPQDPLGAARCVVHGAEFWSQYRINVTEVNPLGASTRLLDVSLQSILRPDPPQGLRVESVPGYPRRLRASWTYPASWPSQPHFLLKFRLQYRPAQHPAWSTVEPAGLEEVITDAVAGLPHAVRVSARDFLDAGTWSTWSPEAWGTPSTGPLQDEIPDWSQGHGQQLEAVVAQEDSPAPARPSLQPDPRPLDHRDPLEQHHHHHHHH

SEQ ID NO: 89 - protein, 348 aa, synthetic construct
  REGION 1..348: note = amino acid sequence of a polypeptide comprising amino acids 24-215 of SEQ ID NO: 82 in which there is a serine at a position corresponding to position 206 of SEQ ID NO: 82 and amino acids 216-363 of SEQ ID NO: 1 and a HIS tag
SPCPQAWGPPGVQYGQPGRPVMLCCPGVSAGTPVSWFRDGDSRLLQGPDSGLGHRLVLAQVDSPDEGTYVCQTLDGVSGGMVTLKLGFPPARPEVSCQAVDYENFSCTWSPGQVSGLPTRYLTSYRKKTLPGAESQRESPSTGPWPCPQDPLEASRCVVHGAEFWSEYRINVTEVNPLGASTSLLDVRLQSILRPDPPQGLRVESVPGYPRRLRASWTYPASWPSQPHFLLKFRLQYRPAQHPAWSTVEPAGLEEVITDAVAGLPHAVRVSARDFLDAGTWSTWSPEAWGTPSTGTIPKEIPAWGQLHTQPEVEPQVDSPAPPRPSLQPHPRLLDHRDSVHHHHHHHH

SEQ ID NO: 90 - protein, 352 aa, synthetic construct
  REGION 1..352: note = amino acid sequence of Mus musculus sIL-11Ra comprising amino acids 24 to 367 of SEQ ID NO: 82 comprising a HIS tag and a serine at a position corresponding to position 206 of SEQ ID NO: 82
SPCPQAWGPPGVQYGQPGRPVMLCCPGVSAGTPVSWFRDGDSRLLQGPDSGLGHRLVLAQVDSPDEGTYVCQTLDGVSGGMVTLKLGFPPARPEVSCQAVDYENFSCTWSPGQVSGLPTRYLTSYRKKTLPGAESQRESPSTGPWPCPQDPLEASRCVVHGAEFWSEYRINVTEVNPLGASTSLLDVRLQSILRPDPPQGLRVESVPGYPRRLHASWTYPASWRRQPHFLLKFRLQYRPAQHPAWSTVEPIGLEEVITDAVAGLPHAVRVSARDFLDAGTWSAWSPEAWGTPSTGPLQDEIPDWSQGHGQQLEAVVAQEDSPAPARPSLQPDPRPLDHRDPLEQHHHHHHHH

SEQ ID NO: 91 - protein, 217 aa, synthetic construct
  REGION 1..217: note = amino acid sequence of light chain of antibody 8E4
QSALTQPPSASGSPGQSVAISCTGTSSDVGGYNFVSWYQQHPGKAPKLLIYEVTKRPSGVPDRFSGSKAGNTASLTVSGLQAEDEADYYCSSYGGSNNAGVFGTGTKVTVLGQPKANPTVTLFPPSSEELQANKATLVCLISDFYPGAVTVAWKADGSPVKAGVETTKPSKQSNNKYAASSYLSLTPEQWKSHRSYSCQVTHEGSTVEKTVAPTECS

SEQ ID NO: 92 - protein, 453 aa, synthetic construct
  REGION 1..453: note = amino acid sequence of heavy chain of antibody 8E4
EVQLLESGGGLVQPGGSLRLSCAASGFTFSWYFMGWVRQAPGKGLEWVSYIYPSGGSTGYADSVKGRFTISRDNSKNTLYLQMHSLRAEDTAVYYCARDEGYCSSTSCYFDAFDIWGQGTMVTVSSASTKGPSVFPLAPCSRSTSESTAALGCLVKDYFPEPVTVSWNSGALTSGVHTFPAVLQSSGLYSLSSVVTVPSSSLGTKTYTCNVDHKPSNTKVDKRVESKYGPPCPPCPAPEFLGGPSVFLFPPKPKDTLMISRTPEVTCVVVDVSQEDPEVQFNWYVDGVEVHNAKTKPREEQFNSTYRVVSVLTVLHQDWLNGKEYKCKVSNKGLPSSIEKTISKAKGQPREPQVYTLPPSQEEMTKNQVSLTCLVKGFYPSDIAVEWESNGQPENNYKTTPPVLDSDGSFFLYSRLTVDKSRWQEGNVFSCSVMHEALHNHYTQKSLSLSLGK

SEQ ID NO: 93 - protein, 214 aa, synthetic construct
  REGION 1..214: note = amino acid sequence of light chain of antibody 8D10
DIQMTQSPSSLSASVGDRVTITCQASQDITNYLNWYLHKPGKAPKLLIYDASNLQTGVPSRFSGSGSGTDFTFTITSLQPEDFGTYYCQQYDTLHPSFGPGTTVDIKRTVAAPSVFIFPPSDEQLKSGTASVVCLLNNFYPREAKVQWKVDNALQSGNSQESVTEQDSKDSTYSLSSTLTLSKADYEKHKVYACEVTHQGLSSPVTKSFNRGEC

SEQ ID NO: 94 - protein, 445 aa, synthetic construct
  REGION 1..445: note = amino acid sequence of heavy chain of antibody 8D10
EVQLLESGGGLVQPGGSLRLSCAASGFTFSRYMMGWVRQAPGKGLEWVSSIVPSGGITIYADSVKGRFTISRDNSKNTLYLQMNSLRAEDTAVYYCARDHMGIVATDWGQGTLVTVSSASTKGPSVFPLAPCSRSTSESTAALGCLVKDYFPEPVTVSWNSGALTSGVHTFPAVLQSSGLYSLSSVVTVPSSSLGTKTYTCNVDHKPSNTKVDKRVESKYGPPCPPCPAPEFLGGPSVFLFPPKPKDTLMISRTPEVTCVVVDVSQEDPEVQFNWYVDGVEVHNAKTKPREEQFNSTYRVVSVLTVLHQDWLNGKEYKCKVSNKGLPSSIEKTISKAKGQPREPQVYTLPPSQEEMTKNQVSLTCLVKGFYPSDIAVEWESNGQPENNYKTTPPVLDSDGSFFLYSRLTVDKSRWQEGNVFSCSVMHEALHNHYTQKSLSLSLGK

SEQ ID NO: 95 - protein, 304 aa, synthetic construct
  REGION 1..304: note = amino acid sequence of SEQ ID NO: 85 comprising a glutamic acid at a position corresponding to position 117 of SEQ ID NO: 1
SSPCPQAWGPPGVQYGQPGRSVKLCCPGVTAGDPVSWFRDGEPKLLQGPDSGLGHELVLAQADSTDEGTYICQTLDGALGGTVTLQLGYPPARPEVSCQAADYENFSCTWSPSQISGLPTRYLTSYRKKTVLGADSQRRSPSTGPWPCPQDPLGAARCVVHGAEFWSQYRINVTEVNPLGASTRLLDVSLQSILRPDPPQGLRVESVPGYPRRLRASWTYPASWPCQPHFLLKFRLQYRPAQHPAWSTVEPAGLEEVITDAVAGLPHAVRVSARDFLDAGTWSTWSPEAWGTPSTGHHHHHHHH

SEQ ID NO: 96 - protein, 304 aa, synthetic construct
  REGION 1..304: note = amino acid sequence of SEQ ID NO: 85 comprising an arginine at a position corresponding to position 66 of SEQ ID NO: 1
SSPCPQAWGPPGVQYGQPGRSVKLCCPGVTAGDPVSWFRDGEPRLLQGPDSGLGHELVLAQADSTDEGTYICQTLDGALGGTVTLQLGYPPARPVVSCQAADYENFSCTWSPSQISGLPTRYLTSYRKKTVLGADSQRRSPSTGPWPCPQDPLGAARCVVHGAEFWSQYRINVTEVNPLGASTRLLDVSLQSILRPDPPQGLRVESVPGYPRRLRASWTYPASWPCQPHFLLKFRLQYRPAQHPAWSTVEPAGLEEVITDAVAGLPHAVRVSARDFLDAGTWSTWSPEAWGTPSTGHHHHHHHH

SEQ ID NO: 97 - protein, 304 aa, synthetic construct
  REGION 1..304: note = amino acid sequence of SEQ ID NO: 85 comprising a serine at a position corresponding to position 65 of SEQ ID NO: 1
SSPCPQAWGPPGVQYGQPGRSVKLCCPGVTAGDPVSWFRDGESKLLQGPDSGLGHELVLAQADSTDEGTYICQTLDGALGGTVTLQLGYPPARPVVSCQAADYENFSCTWSPSQISGLPTRYLTSYRKKTVLGADSQRRSPSTGPWPCPQDPLGAARCVVHGAEFWSQYRINVTEVNPLGASTRLLDVSLQSILRPDPPQGLRVESVPGYPRRLRASWTYPASWPCQPHFLLKFRLQYRPAQHPAWSTVEPAGLEEVITDAVAGLPHAVRVSARDFLDAGTWSTWSPEAWGTPSTGHHHHHHHH

SEQ ID NO: 98 - protein, 304 aa, synthetic construct
  REGION 1..304: note = amino acid sequence of SEQ ID NO: 85 comprising a serine at a position corresponding to position 101 of SEQ ID NO: 1
SSPCPQAWGPPGVQYGQPGRSVKLCCPGVTAGDPVSWFRDGEPKLLQGPDSGLGHELVLAQADSTDEGTYICQTLDGASGGTVTLQLGYPPARPVVSCQAADYENFSCTWSPSQISGLPTRYLTSYRKKTVLGADSQRRSPSTGPWPCPQDPLGAARCVVHGAEFWSQYRINVTEVNPLGASTRLLDVSLQSILRPDPPQGLRVESVPGYPRRLRASWTYPASWPCQPHFLLKFRLQYRPAQHPAWSTVEPAGLEEVITDAVAGLPHAVRVSARDFLDAGTWSTWSPEAWGTPSTGHHHHHHHH

SEQ ID NO: 99 - protein, 304 aa, synthetic construct
  REGION 1..304: note = amino acid sequence of SEQ ID NO: 85 comprising an serine at a position corresponding to position 178 of SEQ ID NO: 1
SSPCPQAWGPPGVQYGQPGRSVKLCCPGVTAGDPVSWFRDGEPKLLQGPDSGLGHELVLAQADSTDEGTYICQTLDGALGGTVTLQLGYPPARPVVSCQAADYENFSCTWSPSQISGLPTRYLTSYRKKTVLGADSQRRSPSTGPWPCPQDPLGASRCVVHGAEFWSQYRINVTEVNPLGASTRLLDVSLQSILRPDPPQGLRVESVPGYPRRLRASWTYPASWPCQPHFLLKFRLQYRPAQHPAWSTVEPAGLEEVITDAVAGLPHAVRVSARDFLDAGTWSTWSPEAWGTPSTGHHHHHHHH

SEQ ID NO: 100 - protein, 400 aa, Homo sapiens
SSPCPQAWGPPGVQYGQPGRSVKLCCPGVTAGDPVSWFRDGEPKLLQGPDSGLGHELVLAQADSTDEGTYICQTLDGALGGTVTLQLGYPPARPVVSCQAADYENFSCTWSPSQISGLPTRYLTSYRKKTVLGADSQRRSPSTGPWPCPQDPLGAARCVVHGAEFWSQYRINVTEVNPLGASTRLLDVSLQSILRPDPPQGLRVESVPGYPRRLRASWTYPASWPCQPHFLLKFRLQYRPAQHPAWSTVEPAGLEEVITDAVAGLPHAVRVSARDFLDAGTWSTWSPEAWGTPSTGTIPKEIPAWGQLHTQPEVEPQVDSPAPPRPSLQPHPRLLDHRDSVEQVAVLASLGILSFLGLVAGALALGLWLRLRRGGKDGSPKPGFLASVIPVDRRPGAPNL

SEQ ID NO: 101 - protein, 410 aa, Macaca fascicularis
SSPCPQAWGPPGVQYGQPGRPVMLCCPGVSAGTPVSWFRDGDSRLLQGPDSGLGHRLVLAQVDSPDEGTYVCQTLDGVSGGMVTLKLGFPPARPEVSCQAVDYENFSCTWSPGQVSGLPTRYLTSYRKKTLPGAESQRESPSTGPWPCPQDPLEASRCVVHGAEFWSEYRINVTEVNPLGASTCLLDVRLQSILRPDPPQGLRVESVPGYPRRLHASWTYPASWRRQPHFLLKFRLQYRPAQHPAWSTVEPIGLEEVITDTVAGLPHAVRVSARDFLDAGTWSAWSPEAWGTPSTGLLQDEIPDWSQGHGQQLEAVVAQEDSLAPARPSLQPDPRPLDHRDPLEQVAVLASLGIFSCLGLAVGALALGLWLRLRRSGKEGPQKPGLLAPMIPVEKLPGIPNLQRTPENFS

SEQ ID NO: 102 - protein, 401 aa, Mus musculus
SPCPQAWGPPGVQYGQPGRPVMLCCPGVSAGTPVSWFRDGDSRLLQGPDSGLGHRLVLAQVDSPDEGTYVCQTLDGVSGGMVTLKLGFPPARPEVSCQAVDYENFSCTWSPGQVSGLPTRYLTSYRKKTLPGAESQRESPSTGPWPCPQDPLEASRCVVHGAEFWSEYRINVTEVNPLGASTCLLDVRLQSILRPDPPQGLRVESVPGYPRRLHASWTYPASWRRQPHFLLKFRLQYRPAQHPAWSTVEPIGLEEVITDTVAGLPHAVRVSARDFLDAGTWSAWSPEAWGTPSTGLLQDEIPDWSQGHGQQLEAVVAQEDSLAPARPSLQPDPRPLDHRDPLEQVAVLASLGIFSCLGLAVGALALGLWLRLRRSGKEGPQKPGLLAPMIPVEKLPGIPNL

SEQ ID NO: 103 - protein, 6 aa, synthetic construct
  REGION 1..6: note = 8E2 L1 consensus sequence
  VARIANT 3: note = X=Y or I or K or M or Q or G or H
VSXYVE

SEQ ID NO: 104 - protein, 6 aa, synthetic construct
  REGION 1..6: note = 8E2 L3.1 consensus sequence
  VARIANT 3: note = X=A or H or F or N or S or W
QQXESQ

SEQ ID NO: 105 - protein, 6 aa, synthetic construct
  REGION 1..6: note = 8E2 L3.2
  VARIANT 4: note = X=A ow W or T or M or Q or W
ETQXPF

SEQ ID NO: 106 - protein, 6 aa, synthetic construct
  REGION 1..6: note = 8E2 H1 consensus sequence
WWWSIT

SEQ ID NO: 107 - protein, 6 aa, synthetic construct
  REGION 1..6: note = 8E2 H2 consensus sequence
VPWGDL

SEQ ID NO: 108 - protein, 6 aa, synthetic construct
  REGION 1..6: note = 8E2 H3.1 consesnsus sequence
  VARIANT 6: note = X=M or R or L
PEDWGX

SEQ ID NO: 109 - protein, 6 aa, synthetic construct
  REGION 1..6: note = 8E2 H3.2 consensus sequence
WGSFWY

SEQ ID NO: 110 - protein, 178 aa, synthetic construct
  REGION 1..178: note = Human PAIDY & W147A IL-11 Mutein
PGPPPGPPRVSPDPRAELDSTVLLTRSLLADTRQLAAQLRDKFPADGDHNLDSLPTLPAIDYALGALQLPGVLTRLRADLLSYLRHVQWLRRAGGSSLKTLEPELGTLQARLDRLLRRLQLLMSRLALPQPPPDPPAPPLAPPSSAAGGIRAAHAILGGLHLTLDWAVRGLLLLKTRL